European Patent Specification EP 3 467 106 B1, published July 9, 2025. Title: Peptide Compound. Applicant: Takeda Pharmaceutical Company Limited. The sequence listing filed with the application follows.

SEQUENCE LISTING (51 sequences)

SEQ ID NO: 1 - protein, 35 aa, Artificial Sequence
  Synthetic Peptide (Formula (I)/(II)/(III))
  MISC_FEATURE (1)..(1): N terminal is modified with P1
  MISC_FEATURE (2)..(2): Xaa stands for Aib
  MISC_FEATURE (6)..(6): alpha-METHYLATION
  MISC_FEATURE (10)..(10): In case of formula (I) and (III), linker alkyl chain as shown in (Gly-Gly-Gly-Gly-X) is linked to epsilon amino group of lysine residue; X = Oda or Pal in formula (I), X=H in formula (III)
  MISC_FEATURE (11)..(11): Xaa stands for Aib, Ala or Ser
  MISC_FEATURE (12)..(12): Xaa stands for Ile or Lys
  MISC_FEATURE (13)..(13): Xaa stands for Aib
  MISC_FEATURE (15)..(15): Xaa stands for Asp or Glu
  MISC_FEATURE (18)..(18): Xaa stands for Ala or Arg
  MISC_FEATURE (20)..(20): Xaa stands for Iva
  MISC_FEATURE (30)..(30): Xaa stands for Aib
  MISC_FEATURE (35)..(35): Xaa stands for Tyr or Phe(2-F)
  MISC_FEATURE (35)..(35): AMIDATION
YXEGTFTSDKXXXLXKQXQXEFVRHLLNKXTRQRX

SEQ ID NO: 2 - protein, 16 aa, Artificial Sequence
  Synthetic Peptide (Reference Example 1)
  MISC_FEATURE (1)..(1): Xaa stands for Iva
  MISC_FEATURE (2)..(15): amino group is protedted at positions 2, 5, 6, 9, 10, 12, 13, 14 and 15
  MISC_FEATURE (11)..(11): Xaa stands for Aib
  MISC_FEATURE (16)..(16): 2-fluoro-l-phenylalanine
XEFVRHLLNKXTRQRF

SEQ ID NO: 3 - protein, 34 aa, Artificial Sequence
  Synthetic Peptide (Reference Example 2)
  MISC_FEATURE (1)..(1): Xaa stands for Aib
  MISC_FEATURE (2)..(33): amino group is protedted at positions 2, 4, 6, 7, 8 ,9, 14, 15, 16, 18, 20, 23, 24, 27, 28, 30, 31, 32 and 33
  MISC_FEATURE (5)..(5): alpha-METHYLATION
  MISC_FEATURE (10)..(10): Xaa stands for Aib
  MISC_FEATURE (12)..(12): Xaa stands for Aib
  MISC_FEATURE (19)..(19): Xaa stands for iva
  MISC_FEATURE (29)..(29): Xaa stands for Aib
  MISC_FEATURE (34)..(34): 2-fluoro-l-phenylalanine
XEGTFTSDKXIXLDKQAQXEFVRHLLNKXTRQRF

SEQ ID NO: 4 - protein, 16 aa, Artificial Sequence
  Synthetic Peptide (Reference Example 3)
  MISC_FEATURE (1)..(1): Xaa stands for Iva
  MISC_FEATURE (2)..(15): amino group is protected at positions 2, 5, 6, 9, 10, 12, 13, 14 and 15
  MISC_FEATURE (11)..(11): Xaa stands for Aib
  MISC_FEATURE (16)..(16): 2-fluoro-l-phenylalanine
XEFVRHLLNKXTRQRF

SEQ ID NO: 5 - protein, 34 aa, Artificial Sequence
  Synthetic Peptide (Reference Example 4)
  MISC_FEATURE (1)..(1): Xaa stands for Aib
  MISC_FEATURE (2)..(33): amino group is protected at positions 2, 4, 6, 7, 8, 9, 14, 15, 16, 17, 18, 20, 23, 24, 27, 28, 30, 31, 32 and 33
  MISC_FEATURE (5)..(5): alpha-METHYLATION
  MISC_FEATURE (10)..(10): Xaa stands for Aib
  MISC_FEATURE (12)..(12): Xaa stands for Aib
  MISC_FEATURE (19)..(19): Xaa stands for Iva
  MISC_FEATURE (29)..(29): Xaa stands for Aib
  MISC_FEATURE (34)..(34): 2-fluoro-l-phenylalanine
XEGTFTSDKXIXLDKQRQXEFVRHLLNKXTRQRF

SEQ ID NO: 6 - protein, 16 aa, Artificial Sequence
  Synthetic Peptide (Reference Example 5)
  MISC_FEATURE (1)..(1): Xaa stands for Iva
  MISC_FEATURE (2)..(16): amino group is protected at positions 2, 5, 6, 9, 10, 12, 13, 14, 15 and 16
  MISC_FEATURE (11)..(11): Xaa stands for Aib
XEFVRHLLNKXTRQRY

SEQ ID NO: 7 - protein, 34 aa, Artificial Sequence
  Synthetic Peptide (Reference Example 6)
  MISC_FEATURE (1)..(1): Xaa stands for Aib
  MISC_FEATURE (2)..(34): amino group is protected at positions 2, 4, 6, 7, 8, 9, 14, 15, 16, 17, 18, 20, 23, 24, 27, 28, 30, 31, 32, 33 and 34
  MISC_FEATURE (5)..(5): alpha-METHYLATION
  MISC_FEATURE (10)..(10): Xaa stands for Aib
  MISC_FEATURE (12)..(12): Xaa stands for Aib
  MISC_FEATURE (19)..(19): Xaa stands for Iva
  MISC_FEATURE (29)..(29): Xaa stands for Aib
XEGTFTSDKXIXLDKQRQXEFVRHLLNKXTRQRY

SEQ ID NO: 8 - protein, 16 aa, Artificial Sequence
  Synthetic Peptide (Reference Example7)
  MISC_FEATURE (1)..(1): Xaa stands for Iva
  MISC_FEATURE (2)..(16): amino group is protected at positions 2, 5, 6, 9, 10, 12, 13, 14, 15 and 16
  MISC_FEATURE (11)..(11): Xaa stands for Aib
XEFVRHLLNKXTRQRY

SEQ ID NO: 9 - protein, 34 aa, Artificial Sequence
  Synthetic Peptide (Reference Example 8)
  MISC_FEATURE (1)..(1): Xaa stands for Aib
  MISC_FEATURE (2)..(34): amino group is protected at positions 2, 4, 6, 7, 8, 9, 14, 15, 16, 18, 20, 23, 24, 27, 28, 30, 31, 32, 33 and 34
  MISC_FEATURE (5)..(5): alpha-METHYLATION
  MISC_FEATURE (10)..(10): Xaa stands for Aib
  MISC_FEATURE (12)..(12): Xaa stands for Aib
  MISC_FEATURE (19)..(19): Xaa stands for Iva
  MISC_FEATURE (29)..(29): Xaa stands for Aib
XEGTFTSDKXIXLDKQAQXEFVRHLLNKXTRQRY

SEQ ID NO: 10 - protein, 35 aa, Artificial Sequence
  Synthetic Peptide (Example 1)
  MISC_FEATURE (2)..(2): Xaa stands for Aib
  MISC_FEATURE (5)..(5): alpha-METHYLATION
  MISC_FEATURE (10)..(10): Linker alkyl chain as shown in (Gly-Gly-Gly-Gly-Pal) is linked to epsilon amino group of lysine
  MISC_FEATURE (11)..(11): Xaa stands for Aib
  MISC_FEATURE (13)..(13): Xaa stands for Aib
  MISC_FEATURE (20)..(20): Xaa stands for Iva
  MISC_FEATURE (30)..(30): Xaa stands for Aib
  MISC_FEATURE (35)..(35): 2-fluoro-l-phenylalanine
YXEGTFTSDKXIXLDKQAQXEFVRHLLNKXTRQRF

SEQ ID NO: 11 - protein, 35 aa, Artificial Sequence; identical to SEQ ID NO: 10
  Synthetic Peptide (Example 2)
  MISC_FEATURE (2)..(2): Xaa stands for Aib
  MISC_FEATURE (5)..(5): alpha-METHYLATION
  MISC_FEATURE (10)..(10): Linker alkyl chain as shown in (Gly-Gly-Gly-Gly-Oda) is linked to epsilon amino group of lysine
  MISC_FEATURE (11)..(11): Xaa stands for Aib
  MISC_FEATURE (13)..(13): Xaa stands for Aib
  MISC_FEATURE (20)..(20): Xaa stands for Iva
  MISC_FEATURE (30)..(30): Xaa stands for Aib
  MISC_FEATURE (35)..(35): 2-fluoro-l-phenylalanine

SEQ ID NO: 12 - protein, 35 aa, Artificial Sequence
  Synthetic Peptide (Example 3)
  MISC_FEATURE (2)..(2): Xaa stands for Aib
  MISC_FEATURE (5)..(5): alpha-METHYLATION
  MISC_FEATURE (10)..(10): Linker alkyl chain as shown in (Gly-Gly-Gly-Gly-Pal) is linked to epsilon amino group of lysine
  MISC_FEATURE (11)..(11): Xaa stands for Aib
  MISC_FEATURE (13)..(13): Xaa stands for Aib
  MISC_FEATURE (20)..(20): Xaa stands for Iva
  MISC_FEATURE (30)..(30): Xaa stands for Aib
  MISC_FEATURE (35)..(35): 2-fluoro-l-phenylalanine
YXEGTFTSDKXIXLDKQRQXEFVRHLLNKXTRQRF

SEQ ID NO: 13 - protein, 35 aa, Artificial Sequence; identical to SEQ ID NO: 12
  Synthetic Peptide (Example 4)
  MISC_FEATURE (2)..(2): Xaa stands for Aib
  MISC_FEATURE (5)..(5): alpha-METHYLATION
  MISC_FEATURE (10)..(10): Linker alkyl chain as shown in (Gly-Gly-Gly-Gly-Oda) is linked to epsilon amino group of lysine
  MISC_FEATURE (11)..(11): Xaa stands for Aib
  MISC_FEATURE (13)..(13): Xaa stands for Aib
  MISC_FEATURE (20)..(20): Xaa stands for Iva
  MISC_FEATURE (30)..(30): Xaa stands for Aib
  MISC_FEATURE (35)..(35): 2-fluoro-l-phenylalanine

SEQ ID NO: 14 - protein, 35 aa, Artificial Sequence; identical to SEQ ID NO: 12
  Synthetic Peptide (Example 5)
  MISC_FEATURE (1)..(1): N-terminal METHYLATION
  MISC_FEATURE (2)..(2): Xaa stands for Aib
  MISC_FEATURE (5)..(5): alpha-METHYLATION
  MISC_FEATURE (10)..(10): Linker alkyl chain as shown in (Gly-Gly-Gly-Gly-Pal) is linked to epsilon amino group of lysine
  MISC_FEATURE (11)..(11): Xaa stands for Aib
  MISC_FEATURE (13)..(13): Xaa stands for Aib
  MISC_FEATURE (20)..(20): Xaa stands for Iva
  MISC_FEATURE (30)..(30): Xaa stands for Aib
  MISC_FEATURE (35)..(35): 2-fluoro-l-phenylalanine

SEQ ID NO: 15 - protein, 35 aa, Artificial Sequence; identical to SEQ ID NO: 12
  Synthetic Peptide (Example 6)
  MISC_FEATURE (1)..(1): N-terminal METHYLATION
  MISC_FEATURE (2)..(2): Xaa stands for Aib
  MISC_FEATURE (5)..(5): alpha-METHYLATION
  MISC_FEATURE (10)..(10): Linker alkyl chain as shown in (Gly-Gly-Gly-Gly-Oda) is linked to epsilon amino group of lysine
  MISC_FEATURE (11)..(11): Xaa stands for Aib
  MISC_FEATURE (13)..(13): Xaa stands for Aib
  MISC_FEATURE (20)..(20): Xaa stands for Iva
  MISC_FEATURE (30)..(30): Xaa stands for Aib
  MISC_FEATURE (35)..(35): 2-fluoro-l-phenylalanine

SEQ ID NO: 16 - protein, 35 aa, Artificial Sequence
  Synthetic Peptide (Example 7)
  MISC_FEATURE (2)..(2): Xaa stands for Aib
  MISC_FEATURE (5)..(5): alpha-METHYLATION
  MISC_FEATURE (10)..(10): Linker alkyl chain as shown in (Gly-Gly-Gly-Gly-Pal) is linked to epsilon amino group of lysine
  MISC_FEATURE (11)..(11): Xaa stands for Aib
  MISC_FEATURE (13)..(13): Xaa stands for Aib
  MISC_FEATURE (20)..(20): Xaa stands for Iva
  MISC_FEATURE (30)..(30): Xaa stands for Aib
YXEGTFTSDKXIXLDKQRQXEFVRHLLNKXTRQRY

SEQ ID NO: 17 - protein, 35 aa, Artificial Sequence; identical to SEQ ID NO: 16
  Synthetic Peptide (Example 8)
  MISC_FEATURE (2)..(2): Xaa stands for Aib
  MISC_FEATURE (5)..(5): alpha-METHYLATION
  MISC_FEATURE (10)..(10): Linker alkyl chain as shown in (Gly-Gly-Gly-Gly-Oda) is linked to epsilon amino group of lysine
  MISC_FEATURE (11)..(11): Xaa stands for Aib
  MISC_FEATURE (13)..(13): Xaa stands for Aib
  MISC_FEATURE (20)..(20): Xaa stands for Aib
  MISC_FEATURE (20)..(20): Xaa stands for Iva
  MISC_FEATURE (30)..(30): Xaa stands for Aib

SEQ ID NO: 18 - protein, 35 aa, Artificial Sequence; identical to SEQ ID NO: 16
  Synthetic Peptide (Example 9)
  MISC_FEATURE (1)..(1): N-terminal METHYLATION
  MISC_FEATURE (2)..(2): Xaa stands for Aib
  MISC_FEATURE (5)..(5): alpha-METHYLATION
  MISC_FEATURE (10)..(10): Linker alkyl chain as shown in (Gly-Gly-Gly-Gly-Pal) is linked to epsilon amino group of lysine
  MISC_FEATURE (11)..(11): Xaa stands for Aib
  MISC_FEATURE (13)..(13): Xaa stands for Aib
  MISC_FEATURE (20)..(20): Xaa stands for Iva
  MISC_FEATURE (30)..(30): Xaa stands for Aib

SEQ ID NO: 19 - protein, 35 aa, Artificial Sequence; identical to SEQ ID NO: 16
  Synthetic Peptide (Example 10)
  MISC_FEATURE (1)..(1): N-terminal METHYLATION
  MISC_FEATURE (2)..(2): Xaa stands for Aib
  MISC_FEATURE (5)..(5): alpha-METHYLATION
  MISC_FEATURE (10)..(10): Linker alkyl chain as shown in (Gly-Gly-Gly-Gly-Oda) is linked to epsilon amino group of lysine
  MISC_FEATURE (11)..(11): Xaa stands for Aib
  MISC_FEATURE (13)..(13): Xaa stands for Aib
  MISC_FEATURE (20)..(20): Xaa stands for Iva
  MISC_FEATURE (30)..(30): Xaa stands for Aib

SEQ ID NO: 20 - protein, 35 aa, Artificial Sequence
  Synthetic Peptide (Example 11)
  MISC_FEATURE (2)..(2): Xaa stands for Aib
  MISC_FEATURE (5)..(5): alpha-METHYLATION
  MISC_FEATURE (10)..(10): Linker alkyl chain as shown in (Gly-Gly-Gly-Gly-Pal) is linked to epsilon amino group of lysine
  MISC_FEATURE (13)..(13): Xaa stands for Aib
  MISC_FEATURE (20)..(20): Xaa stands for Iva
  MISC_FEATURE (30)..(30): Xaa stands for Aib
YXEGTFTSDKAIXLDKQRQXEFVRHLLNKXTRQRY

SEQ ID NO: 21 - protein, 35 aa, Artificial Sequence; identical to SEQ ID NO: 20
  Synthetic Peptide (Example 12)
  MISC_FEATURE (2)..(2): Xaa stands for Aib
  MISC_FEATURE (5)..(5): alpha-METHYLATION
  MISC_FEATURE (10)..(10): Linker alkyl chain as shown in (Gly-Gly-Gly-Gly-Oda) is linked to epsilon amino group of lysine
  MISC_FEATURE (13)..(13): Xaa stands for Aib
  MISC_FEATURE (20)..(20): Xaa stands for Iva
  MISC_FEATURE (30)..(30): Xaa stands for Aib

SEQ ID NO: 22 - protein, 35 aa, Artificial Sequence; identical to SEQ ID NO: 20
  Synthetic Peptide (Example 13)
  MISC_FEATURE (1)..(1): N-terminal METHYLATION
  MISC_FEATURE (2)..(2): Xaa stands for Aib
  MISC_FEATURE (5)..(5): alpha-METHYLATION
  MISC_FEATURE (10)..(10): Linker alkyl chain as shown in (Gly-Gly-Gly-Gly-Pal) is linked to epsilon amino group of lysine
  MISC_FEATURE (13)..(13): Xaa stands for Aib
  MISC_FEATURE (20)..(20): Xaa stands for Iva
  MISC_FEATURE (30)..(30): Xaa stands for Aib

SEQ ID NO: 23 - protein, 35 aa, Artificial Sequence; identical to SEQ ID NO: 20
  Synthetic Peptide (Example 14)
  MISC_FEATURE (1)..(1): N-terminal METHYLATION
  MISC_FEATURE (2)..(2): Xaa stands for Aib
  MISC_FEATURE (5)..(5): alpha-METHYLATION
  MISC_FEATURE (10)..(10): Linker alkyl chain as shown in (Gly-Gly-Gly-Gly-Oda) is linked to epsilon amino group of lysine
  MISC_FEATURE (13)..(13): Xaa stands for Aib
  MISC_FEATURE (20)..(20): Xaa stands for Iva
  MISC_FEATURE (30)..(30): Xaa stands for Aib

SEQ ID NO: 24 - protein, 35 aa, Artificial Sequence
  Synthetic Peptide (Example 15)
  MISC_FEATURE (2)..(2): Xaa stands for Aib
  MISC_FEATURE (5)..(5): alpha-METHYLATION
  MISC_FEATURE (10)..(10): Linker alkyl chain as shown in (Gly-Gly-Gly-Gly-Pal) is linked to epsilon amino group of lysine
  MISC_FEATURE (13)..(13): Xaa stands for Aib
  MISC_FEATURE (20)..(20): Xaa stands for Iva
  MISC_FEATURE (30)..(30): Xaa stands for Aib
YXEGTFTSDKSIXLDKQRQXEFVRHLLNKXTRQRY

SEQ ID NO: 25 - protein, 35 aa, Artificial Sequence; identical to SEQ ID NO: 24
  Synthetic Peptide (Example 16)
  MISC_FEATURE (2)..(2): Xaa stands for Aib
  MISC_FEATURE (5)..(5): alpha-METHYLATION
  MISC_FEATURE (10)..(10): Linker alkyl chain as shown in (Gly-Gly-Gly-Gly-Oda) is linked to epsilon amino group of lysine
  MISC_FEATURE (13)..(13): Xaa stands for Aib
  MISC_FEATURE (20)..(20): Xaa stands for Iva
  MISC_FEATURE (30)..(30): Xaa stands for Aib

SEQ ID NO: 26 - protein, 35 aa, Artificial Sequence; identical to SEQ ID NO: 24
  Synthetic Peptide (Example 17)
  MISC_FEATURE (1)..(1): N-terminal METHYLATION
  MISC_FEATURE (2)..(2): Xaa stands for Aib
  MISC_FEATURE (5)..(5): alpha-METHYLATION
  MISC_FEATURE (10)..(10): Linker alkyl chain as shown in (Gly-Gly-Gly-Gly-Pal) is linked to epsilon amino group of lysine
  MISC_FEATURE (13)..(13): Xaa stands for Aib
  MISC_FEATURE (20)..(20): Xaa stands for Iva
  MISC_FEATURE (30)..(30): Xaa stands for Aib

SEQ ID NO: 27 - protein, 35 aa, Artificial Sequence; identical to SEQ ID NO: 24
  Synthetic Peptide (Example 18)
  MISC_FEATURE (1)..(1): N-terminal METHYLATION
  MISC_FEATURE (2)..(2): Xaa stands for Aib
  MISC_FEATURE (5)..(5): alpha-METHYLATION
  MISC_FEATURE (10)..(10): Linker alkyl chain as shown in (Gly-Gly-Gly-Gly-Oda) is linked to epsilon amino group of lysine
  MISC_FEATURE (13)..(13): Xaa stands for Aib
  MISC_FEATURE (20)..(20): Xaa stands for Iva
  MISC_FEATURE (30)..(30): Xaa stands for Aib

SEQ ID NO: 28 - protein, 35 aa, Artificial Sequence
  Synthetic Peptide (Example 19)
  MISC_FEATURE (2)..(2): Xaa stands for Aib
  MISC_FEATURE (5)..(5): alpha-METHYLATION
  MISC_FEATURE (10)..(10): Linker alkyl chain as shown in (Gly-Gly-Gly-Gly-Pal) is linked to epsilon amino group of lysine
  MISC_FEATURE (11)..(11): Xaa stands for Aib
  MISC_FEATURE (13)..(13): Xaa stands for Aib
  MISC_FEATURE (20)..(20): Xaa stands for Iva
  MISC_FEATURE (30)..(30): Xaa stands for Aib
YXEGTFTSDKXKXLDKQRQXEFVRHLLNKXTRQRY

SEQ ID NO: 29 - protein, 35 aa, Artificial Sequence; identical to SEQ ID NO: 28
  Synthetic Peptide (Example 20)
  MISC_FEATURE (2)..(2): Xaa stands for Aib
  MISC_FEATURE (5)..(5): alpha-METHYLATION
  MISC_FEATURE (10)..(10): Linker alkyl chain as shown in (Gly-Gly-Gly-Gly-Oda) is linked to epsilon amino group of lysine
  MISC_FEATURE (11)..(11): Xaa stands for Aib
  MISC_FEATURE (13)..(13): Xaa stands for Aib
  MISC_FEATURE (20)..(20): Xaa stands for Iva
  MISC_FEATURE (30)..(30): Xaa stands for Aib

SEQ ID NO: 30 - protein, 35 aa, Artificial Sequence; identical to SEQ ID NO: 28
  Synthetic Peptide (Example 21)
  MISC_FEATURE (1)..(1): N-terminal METHYLATION
  MISC_FEATURE (2)..(2): Xaa stands for Aib
  MISC_FEATURE (5)..(5): alpha-METHYLATION
  MISC_FEATURE (10)..(10): Linker alkyl chain as shown in (Gly-Gly-Gly-Gly-Pal) is linked to epsilon amino group of lysine
  MISC_FEATURE (11)..(11): Xaa stands for Aib
  MISC_FEATURE (13)..(13): Xaa stands for Aib
  MISC_FEATURE (20)..(20): Xaa stands for Iva
  MISC_FEATURE (30)..(30): Xaa stands for Aib

SEQ ID NO: 31 - protein, 34 aa, Artificial Sequence
  Synthetic Peptide (Example 22)
  MISC_FEATURE (1)..(1): N-terminal METHYLATION
  MISC_FEATURE (2)..(2): Xaa stands for Aib
  MISC_FEATURE (5)..(5): alpha-METHYLATION
  MISC_FEATURE (10)..(10): Linker alkyl chain as shown in (Gly-Gly-Gly-Gly-Oda) is linked to epsilon amino group of lysine
  MISC_FEATURE (11)..(11): Xaa stands for Aib
  MISC_FEATURE (13)..(13): Xaa stands for Aib
  MISC_FEATURE (20)..(20): Xaa stands for Iva
  MISC_FEATURE (30)..(30): Xaa stands for Aib
YXEGTFTSDKXKXLDKQRQXEFVRHLLNKXTRQR

SEQ ID NO: 32 - protein, 35 aa, Artificial Sequence
  Synthetic Peptide (Example 23)
  MISC_FEATURE (2)..(2): Xaa stands for Aib
  MISC_FEATURE (5)..(5): alpha-METHYLATION
  MISC_FEATURE (10)..(10): Linker alkyl chain as shown in (Gly-Gly-Gly-Gly-Pal) is linked to epsilon amino group of lysine
  MISC_FEATURE (13)..(13): Xaa stands for Aib
  MISC_FEATURE (20)..(20): Xaa stands for Iva
  MISC_FEATURE (30)..(30): Xaa stands for Aib
YXEGTFTSDKSKXLDKQRQXEFVRHLLNKXTRQRY

SEQ ID NO: 33 - protein, 35 aa, Artificial Sequence; identical to SEQ ID NO: 32
  Synthetic Peptide (Example 24)
  MISC_FEATURE (2)..(2): Xaa stands for Aib
  MISC_FEATURE (5)..(5): alpha-METHYLATION
  MISC_FEATURE (10)..(10): Linker alkyl chain as shown in (Gly-Gly-Gly-Gly-Oda) is linked to epsilon amino group of lysine
  MISC_FEATURE (13)..(13): Xaa stands for Aib
  MISC_FEATURE (20)..(20): Xaa stands for Iva
  MISC_FEATURE (30)..(30): Xaa stands for Aib

SEQ ID NO: 34 - protein, 35 aa, Artificial Sequence; identical to SEQ ID NO: 32
  Synthetic Peptide (Example 25)
  MISC_FEATURE (1)..(1): N-terminal METHYLATION
  MISC_FEATURE (2)..(2): Xaa stands for Aib
  MISC_FEATURE (5)..(5): alpha-METHYLATION
  MISC_FEATURE (10)..(10): Linker alkyl chain as shown in (Gly-Gly-Gly-Gly-Pal) is linked to epsilon amino group of lysine
  MISC_FEATURE (13)..(13): Xaa stands for Aib
  MISC_FEATURE (20)..(20): Xaa stands for Iva
  MISC_FEATURE (30)..(30): Xaa stands for Aib

SEQ ID NO: 35 - protein, 35 aa, Artificial Sequence; identical to SEQ ID NO: 32
  Synthetic Peptide (Example 26)
  MISC_FEATURE (1)..(1): N-terminal METHYLATION
  MISC_FEATURE (2)..(2): Xaa stands for Aib
  MISC_FEATURE (5)..(5): alpha-METHYLATION
  MISC_FEATURE (10)..(10): Linker alkyl chain as shown in (Gly-Gly-Gly-Gly-Oda) is linked to epsilon amino group of lysine
  MISC_FEATURE (13)..(13): Xaa stands for Aib
  MISC_FEATURE (20)..(20): Xaa stands for Iva
  MISC_FEATURE (30)..(30): Xaa stands for Aib

SEQ ID NO: 36 - protein, 35 aa, Artificial Sequence
  Synthetic Peptide (Example 27)
  MISC_FEATURE (2)..(2): Xaa stands for Aib
  MISC_FEATURE (5)..(5): alpha-METHYLATION
  MISC_FEATURE (10)..(10): Linker alkyl chain as shown in (Gly-Gly-Gly-Gly-Pal) is linked to epsilon amino group of lysine
  MISC_FEATURE (11)..(11): Xaa stands for Aib
  MISC_FEATURE (13)..(13): Xaa stands for Aib
  MISC_FEATURE (20)..(20): Xaa stands for Iva
  MISC_FEATURE (30)..(30): Xaa stands for Aib
YXEGTFTSDKXIXLDKQAQXEFVRHLLNKXTRQRY

SEQ ID NO: 37 - protein, 35 aa, Artificial Sequence; identical to SEQ ID NO: 36
  Synthetic Peptide (Example 28)
  MISC_FEATURE (2)..(2): Xaa stands for Aib
  MISC_FEATURE (5)..(5): alpha-METHYLATION
  MISC_FEATURE (10)..(10): Linker alkyl chain as shown in (Gly-Gly-Gly-Gly-Oda) is linked to epsilon amino group of lysine
  MISC_FEATURE (11)..(11): Xaa stands for Aib
  MISC_FEATURE (13)..(13): Xaa stands for Aib
  MISC_FEATURE (20)..(20): Xaa stands for Iva
  MISC_FEATURE (30)..(30): Xaa stands for Aib

SEQ ID NO: 38 - protein, 35 aa, Artificial Sequence; identical to SEQ ID NO: 36
  Synthetic Peptide (Example 29)
  MISC_FEATURE (1)..(1): N-terminal METHYLATION
  MISC_FEATURE (2)..(2): Xaa stands for Aib
  MISC_FEATURE (5)..(5): alpha-METHYLATION
  MISC_FEATURE (10)..(10): Linker alkyl chain as shown in (Gly-Gly-Gly-Gly-Pal) is linked to epsilon amino group of lysine
  MISC_FEATURE (11)..(11): Xaa stands for Aib
  MISC_FEATURE (13)..(13): Xaa stands for Aib
  MISC_FEATURE (20)..(20): Xaa stands for Iva
  MISC_FEATURE (30)..(30): Xaa stands for Aib

SEQ ID NO: 39 - protein, 35 aa, Artificial Sequence; identical to SEQ ID NO: 36
  Synthetic Peptide (Example 30)
  MISC_FEATURE (1)..(1): N-terminal METHYLATION
  MISC_FEATURE (2)..(2): Xaa stands for Aib
  MISC_FEATURE (5)..(5): alpha-METHYLATION
  MISC_FEATURE (10)..(10): Linker alkyl chain as shown in (Gly-Gly-Gly-Gly-Oda) is linked to epsilon amino group of lysine
  MISC_FEATURE (11)..(11): Xaa stands for Aib
  MISC_FEATURE (13)..(13): Xaa stands for Aib
  MISC_FEATURE (20)..(20): Xaa stands for Iva
  MISC_FEATURE (30)..(30): Xaa stands for Aib

SEQ ID NO: 40 - protein, 35 aa, Artificial Sequence
  Synthetic Peptide (Example 31)
  MISC_FEATURE (2)..(2): Xaa stands for Aib
  MISC_FEATURE (5)..(5): alpha-METHYLATION
  MISC_FEATURE (10)..(10): Linker alkyl chain as shown in (Gly-Gly-Gly-Gly-Pal) is linked to epsilon amino group of lysine
  MISC_FEATURE (11)..(11): Xaa stands for Aib
  MISC_FEATURE (13)..(13): Xaa stands for Aib
  MISC_FEATURE (20)..(20): Xaa stands for Iva
  MISC_FEATURE (30)..(30): Xaa stands for Aib
YXEGTFTSDKXIXLEKQRQXEFVRHLLNKXTRQRY

SEQ ID NO: 41 - protein, 35 aa, Artificial Sequence; identical to SEQ ID NO: 40
  Synthetic Peptide (Example 32)
  MISC_FEATURE (2)..(2): Xaa stands for Aib
  MISC_FEATURE (5)..(5): alpha-METHYLATION
  MISC_FEATURE (10)..(10): Linker alkyl chain as shown in (Gly-Gly-Gly-Gly-Oda) is linked to epsilon amino group of lysine
  MISC_FEATURE (11)..(11): Xaa stands for Aib
  MISC_FEATURE (13)..(13): Xaa stands for Aib
  MISC_FEATURE (20)..(20): Xaa stands for Iva
  MISC_FEATURE (30)..(30): Xaa stands for Aib

SEQ ID NO: 42 - protein, 35 aa, Artificial Sequence; identical to SEQ ID NO: 40
  Synthetic Peptide (Example 33)
  MISC_FEATURE (1)..(1): N-terminal METHYLATION
  MISC_FEATURE (2)..(2): Xaa stands for Aib
  MISC_FEATURE (5)..(5): alpha-METHYLATION
  MISC_FEATURE (10)..(10): Linker alkyl chain as shown in (Gly-Gly-Gly-Gly-Pal) is linked to epsilon amino group of lysine
  MISC_FEATURE (11)..(11): Xaa stands for Aib
  MISC_FEATURE (13)..(13): Xaa stands for Aib
  MISC_FEATURE (20)..(20): Xaa stands for Iva
  MISC_FEATURE (30)..(30): Xaa stands for Aib

SEQ ID NO: 43 - protein, 35 aa, Artificial Sequence; identical to SEQ ID NO: 40
  Synthetic Peptide (Example 34)
  MISC_FEATURE (1)..(1): N-terminal METHYLATION
  MISC_FEATURE (2)..(2): Xaa stands for Aib
  MISC_FEATURE (5)..(5): alpha-METHYLATION
  MISC_FEATURE (10)..(10): Linker alkyl chain as shown in (Gly-Gly-Gly-Gly-Oda) is linked to epsilon amino group of lysine
  MISC_FEATURE (11)..(11): Xaa stands for Aib
  MISC_FEATURE (13)..(13): Xaa stands for Aib
  MISC_FEATURE (20)..(20): Xaa stands for Iva
  MISC_FEATURE (30)..(30): Xaa stands for Aib

SEQ ID NO: 44 - protein, 35 aa, Artificial Sequence
  Synthetic Peptide (Example 35)
  MISC_FEATURE (2)..(2): Xaa stands for Aib
  MISC_FEATURE (5)..(5): alpha-METHYLATION
  MISC_FEATURE (10)..(10): Linker alkyl chain as shown in (Gly-Gly-Gly-Gly-Pal) is linked to epsilon amino group of lysine
  MISC_FEATURE (13)..(13): Xaa stands for Aib
  MISC_FEATURE (20)..(20): Xaa stands for Iva
  MISC_FEATURE (30)..(30): Xaa stands for Aib
YXEGTFTSDKAIXLEKQRQXEFVRHLLNKXTRQRY

SEQ ID NO: 45 - protein, 35 aa, Artificial Sequence; identical to SEQ ID NO: 44
  Synthetic Peptide (Example 36)
  MISC_FEATURE (2)..(2): Xaa stands for Aib
  MISC_FEATURE (5)..(5): alpha-METHYLATION
  MISC_FEATURE (10)..(10): Linker alkyl chain as shown in (Gly-Gly-Gly-Gly-Oda) is linked to epsilon amino group of lysine
  MISC_FEATURE (13)..(13): Xaa stands for Aib
  MISC_FEATURE (20)..(20): Xaa stands for Iva
  MISC_FEATURE (30)..(30): Xaa stands for Aib

SEQ ID NO: 46 - protein, 35 aa, Artificial Sequence; identical to SEQ ID NO: 44
  Synthetic Peptide (Example 37)
  MISC_FEATURE (1)..(1): N-terminal METHYLATION
  MISC_FEATURE (2)..(2): Xaa stands for Aib
  MISC_FEATURE (5)..(5): alpha-METHYLATION
  MISC_FEATURE (10)..(10): Linker alkyl chain as shown in (Gly-Gly-Gly-Gly-Pal) is linked to epsilon amino group of lysine
  MISC_FEATURE (13)..(13): Xaa stands for Aib
  MISC_FEATURE (20)..(20): Xaa stands for Iva
  MISC_FEATURE (30)..(30): Xaa stands for Aib

SEQ ID NO: 47 - protein, 35 aa, Artificial Sequence; identical to SEQ ID NO: 44
  Synthetic Peptide (Example 38)
  MISC_FEATURE (1)..(1): N-terminal METHYLATION
  MISC_FEATURE (2)..(2): Xaa stands for Aib
  MISC_FEATURE (5)..(5)
  MISC_FEATURE (10)..(10): Linker alkyl chain as shown in (Gly-Gly-Gly-Gly-Oda) is linked to epsilon amino group of lysine
  MISC_FEATURE (13)..(13): Xaa stands for Aib
  MISC_FEATURE (20)..(20): Xaa stands for Iva
  MISC_FEATURE (30)..(30): Xaa stands for Aib

SEQ ID NO: 48 - protein, 35 aa, Artificial Sequence
  Synthetic Peptide (Example 39)
  MISC_FEATURE (2)..(2): Xaa stands for Aib
  MISC_FEATURE (5)..(5): alpha-METHYLATION
  MISC_FEATURE (10)..(10): Linker alkyl chain as shown in (Gly-Gly-Gly-Gly-Pal) is linked to epsilon amino group of lysine
  MISC_FEATURE (13)..(13): Xaa stands for Aib
  MISC_FEATURE (20)..(20): Xaa stands for Iva
  MISC_FEATURE (30)..(30): Xaa stands for Aib
YXEGTFTSDKSIXLEKQRQXEFVRHLLNKXTRQRY

SEQ ID NO: 49 - protein, 35 aa, Artificial Sequence; identical to SEQ ID NO: 48
  Synthetic Peptide (Example 40)
  MISC_FEATURE (2)..(2): Xaa stands for Aib
  MISC_FEATURE (5)..(5): alpha-METHYLATION
  MISC_FEATURE (10)..(10): Linker alkyl chain as shown in (Gly-Gly-Gly-Gly-Oda) is linked to epsilon amino group of lysine
  MISC_FEATURE (13)..(13): Xaa stands for Aib
  MISC_FEATURE (20)..(20): Xaa stands for Iva
  MISC_FEATURE (30)..(30): Xaa stands for Aib

SEQ ID NO: 50 - protein, 35 aa, Artificial Sequence; identical to SEQ ID NO: 48
  Synthetic Peptide (Example 41)
  MISC_FEATURE (1)..(1): N-terminal METHYLATION
  MISC_FEATURE (2)..(2): Xaa stands for Aib
  MISC_FEATURE (5)..(5): alpha-METHYLATION
  MISC_FEATURE (10)..(10): Linker alkyl chain as shown in (Gly-Gly-Gly-Gly-Pal) is linked to epsilon amino group of lysine
  MISC_FEATURE (13)..(13): Xaa stands for Aib
  MISC_FEATURE (20)..(20): Xaa stands for Iva
  MISC_FEATURE (30)..(30): Xaa stands for Aib

SEQ ID NO: 51 - protein, 35 aa, Artificial Sequence; identical to SEQ ID NO: 48
  Synthetic Peptide (Example 42)
  MISC_FEATURE (1)..(1): N-terminal METHYLATION
  MISC_FEATURE (2)..(2): Xaa stands for Aib
  MISC_FEATURE (5)..(5): alpha-METHYLATION
  MISC_FEATURE (10)..(10): Linker alkyl chain as shown in (Gly-Gly-Gly-Gly-Oda) is linked to epsilon amino group of lysine
  MISC_FEATURE (13)..(13): Xaa stands for Aib
  MISC_FEATURE (20)..(20): Xaa stands for Iva
  MISC_FEATURE (30)..(30): Xaa stands for Aib